European Patent Application EP 4 389 902 A1, published June 26, 2024. Title: Method for preparing human artificial chromosome vector in human cell. Applicant: National University Corporation Tottori University. The sequence listing filed with the application follows.

SEQUENCE LISTING (18 sequences)

SEQ ID NO: 1 - DNA, 20 bp, Homo sapiens
  source 1..20: mol_type = unassigned DNA
gacaggtaaggattactagg

SEQ ID NO: 2 - DNA, 20 bp, Homo sapiens
  source 1..20: mol_type = unassigned DNA
taaagatgtgctccttcccg

SEQ ID NO: 3 - DNA, 20 bp, Homo sapiens
  source 1..20: mol_type = unassigned DNA
agaactgaagcatcactcac

SEQ ID NO: 4 - DNA, 20 bp, Homo sapiens
  source 1..20: mol_type = unassigned DNA
agaagcgaatcctgcttgca

SEQ ID NO: 5 - DNA, 23 bp, Homo sapiens
  source 1..23: mol_type = unassigned DNA
gacaggtaaggattactaggagg

SEQ ID NO: 6 - DNA, 23 bp, Homo sapiens
  source 1..23: mol_type = unassigned DNA
taaagatgtgctccttcccgagg

SEQ ID NO: 7 - DNA, 20 bp, synthetic construct
  misc_feature 1..20: note = primer
  source 1..20: mol_type = other DNA
aactgagcccctttcttcgg

SEQ ID NO: 8 - DNA, 20 bp, synthetic construct
  misc_feature 1..20: note = primer
  source 1..20: mol_type = other DNA
aggattctctgctcccccat

SEQ ID NO: 9 - DNA, 22 bp, synthetic construct
  misc_feature 1..22: note = primer
  source 1..22: mol_type = other DNA
gtgcaactgtcagaccaaaaca

SEQ ID NO: 10 - DNA, 21 bp, synthetic construct
  misc_feature 1..21: note = primer
  source 1..21: mol_type = other DNA
tgcctgactgaaaagatgagt

SEQ ID NO: 11 - DNA, 20 bp, synthetic construct
  misc_feature 1..20: note = primer
  source 1..20: mol_type = other DNA
tgacaggcatccatgggaac

SEQ ID NO: 12 - DNA, 20 bp, synthetic construct
  misc_feature 1..20: note = primer
  source 1..20: mol_type = other DNA
ctcagacccggagctttctc

SEQ ID NO: 13 - DNA, 20 bp, synthetic construct
  misc_feature 1..20: note = primer
  source 1..20: mol_type = other DNA
ggctccatcccatgtgagag

SEQ ID NO: 14 - DNA, 23 bp, synthetic construct
  misc_feature 1..23: note = primer
  source 1..23: mol_type = other DNA
agaactgaagcatcactcactgg

SEQ ID NO: 15 - DNA, 20 bp, Homo sapiens
  source 1..20: mol_type = unassigned DNA
agactgtagccttgacccag

SEQ ID NO: 16 - DNA, 20 bp, Homo sapiens
  source 1..20: mol_type = unassigned DNA
ctgtggacgtattaacttac

SEQ ID NO: 17 - DNA, 20 bp, synthetic construct
  misc_feature 1..20: note = primer
  source 1..20: mol_type = other DNA
tgtgcaaccagctttggaac

SEQ ID NO: 18 - DNA, 23 bp, synthetic construct
  misc_feature 1..23: note = primer
  source 1..23: mol_type = other DNA
accattagaggactctgtcagtg